European Patent Specification EP 3 553 170 B1, published February 14, 2024. Title: SUBSTANTIALLY PURE HUMAN RETINAL PROGENITOR, FOREBRAIN PROGENITOR, AND RETINAL PIGMENT EPITHELIUM CELL CULTURES AND METHODS OF MAKING THE SAME. Applicant: Wisconsin Alumni Research Foundation. The sequence listing filed with the application follows.

SEQUENCE LISTING (60 sequences)

SEQ ID NO: 1 - DNA, 20 bp, Artificial Sequence
  Synthetic oligonucleotide
agaacctgtcacaagctgtg

SEQ ID NO: 2 - DNA, 20 bp, Artificial Sequence
  Synthetic oligonucleotide
gacagcaagctgaggatgtc

SEQ ID NO: 3 - DNA, 20 bp, Artificial Sequence
  Synthetic oligonucleotide
gcgagaagatgacccagatc

SEQ ID NO: 4 - DNA, 19 bp, Artificial Sequence
  Synthetic oligonucleotide
ccagtggtacggccagagg

SEQ ID NO: 5 - DNA, 24 bp, Artificial Sequence
  Synthetic oligonucleotide
atttataggctggccctcacggaa

SEQ ID NO: 6 - DNA, 24 bp, Artificial Sequence
  Synthetic olionucleotide
tgttctgccggagtcataaagcct

SEQ ID NO: 7 - DNA, 20 bp, Artificial Sequence
  Synthetic oligonucleotide
acccagttcatagcggtgac

SEQ ID NO: 8 - DNA, 20 bp, Artificial Sequence
  Synthetic oligonucleotide
caattgtcatgggattgcag

SEQ ID NO: 9 - DNA, 24 bp, Artificial Sequence
  Synthetic oligonuleotide
attcaacgaagcccactacccaga

SEQ ID NO: 10 - DNA, 24 bp, Artificial Sequence
  Synthetic oligonucleotide
atccttggctgacttgaggatgga

SEQ ID NO: 11 - DNA, 21 bp, Artificial Sequence
  Synthetic oligonucleotide
ggcgacacaggacaatcttta

SEQ ID NO: 12 - DNA, 19 bp, Artificial Sequence
  Synthetic oligonucleotide
ttccggcagctccgttttc

SEQ ID NO: 13 - DNA, 24 bp, Artificial Sequence
  Synthetic oligonucleotide
tattctgtcaacgccttggcccta

SEQ ID NO: 14 - DNA, 24 bp, Artificial Sequence
  Synthetic oligonucleotide
tgcatttagccctccggttcttga

SEQ ID NO: 15 - DNA, 24 bp, Artificial Sequence
  Synthetic oligonucleotide
agcaccttggatgggtattccaga

SEQ ID NO: 16 - DNA, 24 bp, Artificial Sequence
  Synthetic oligonucleotide
acacaatcctgaggcacagtctga

SEQ ID NO: 17 - DNA, 20 bp, Artificial Sequence
  Synthetic oligonucleotide
ccctggtttctctgggactt

SEQ ID NO: 18 - DNA, 20 bp, Artificial Sequence
  Synthetic oligonucleotide
gcagtctgtggggtcgtatt

SEQ ID NO: 19 - DNA, 20 bp, Artificial Sequence
  Synthetic oligonucleotide
accacagtccatgccatcac

SEQ ID NO: 20 - DNA, 20 bp, Artificial Sequence
  Synthetic oligonucleotide
tccaccaccctgttgctgta

SEQ ID NO: 21 - DNA, 20 bp, Artificial Sequence
  Synthetic oligonucleotide
gcaaagagcccgtcgtctac

SEQ ID NO: 22 - DNA, 20 bp, Artificial Sequence
  Synthetic oligonucleotide
cgtgtcaggtagcggttgta

SEQ ID NO: 23 - DNA, 20 bp, Artificial Sequence
  Synthetic oligonucleotide
caagatctcggaccgctact

SEQ ID NO: 24 - DNA, 20 bp, Artificial Sequence
  Synthetic oligonucleotide
ccgtggtcagcatcttgtta

SEQ ID NO: 25 - DNA, 24 bp, Artificial Sequence
  Synthetic oligonucleotide
ttcacgagcgtcctgtatgcagat

SEQ ID NO: 26 - DNA, 24 bp, Artificial Sequence
  Synthetic oligonucleotide
ttgcaaagcaggatccatcaagcc

SEQ ID NO: 27 - DNA, 20 bp, Artificial Sequence
  Synthetic oligonucleotide
caaaggcaaacaacccactt

SEQ ID NO: 28 - DNA, 20 bp, Artificial Sequence
  Synthetic oligonucleotide
tctgctggaggctgaggtat

SEQ ID NO: 29 - DNA, 24 bp, Artificial Sequence
  Synthetic oligonucleotide
ccatcatttccgagtgcaagtgct

SEQ ID NO: 30 - DNA, 24 bp, Artificial Sequence
  Synthetic oligonucleotide
aagctaggtctctgtagcccagaa

SEQ ID NO: 31 - DNA, 24 bp, Artificial Sequence
  Synthetic oligonucleotide
cgagcaatttgccaagctcctgaa

SEQ ID NO: 32 - DNA, 24 bp, Artificial Sequence
  Synthetic oligonucleotide
ttcgggcactgcaggaacaaattc

SEQ ID NO: 33 - DNA, 20 bp, Artificial Sequence
  Synthetic oligonucleotide
gtggaggaagctgacaacaa

SEQ ID NO: 34 - DNA, 20 bp, Artificial Sequence
  Synthetic oligonucleotide
attctccaggttgcctctca

SEQ ID NO: 35 - DNA, 24 bp, Artificial Sequence
  Synthetic oligonucleotide
tacctggaccattggtattggcgt

SEQ ID NO: 36 - DNA, 24 bp, Artificial Sequence
  Synthetic oligonucleotide
taagtccagcccatggttacggtt

SEQ ID NO: 37 - DNA, 20 bp, Artificial Sequence
  Synthetic oligonucleotide
caacagcagaatggaggtca

SEQ ID NO: 38 - DNA, 22 bp, Artificial Sequence
  Synthetic oligonucleotide
ctgggtggaaagagagaagctg

SEQ ID NO: 39 - DNA, 20 bp, Artificial Sequence
  Synthetic oligonucleotide
cggagtgaatcagctcggtg

SEQ ID NO: 40 - DNA, 23 bp, Artificial Sequence
  Synthetic oligonucleotide
ccgcttatactgggctattttgc

SEQ ID NO: 41 - DNA, 24 bp, Artificial Sequence
  Synthetic oligonucleotide
agtgaatcagctcggtggtgtctt

SEQ ID NO: 42 - DNA, 24 bp, Artificial Sequence
  Synthetic oligonucleotide
tgcagaattcgggaaatgtcgcac

SEQ ID NO: 43 - DNA, 21 bp, Artificial Sequence
  Synthetic oligonucleotide
ctcggtggtgtctttgtcaac

SEQ ID NO: 44 - DNA, 21 bp, Artificial Sequence
  Synthetic oligonucleotide
acttttgcatctgcatgggtc

SEQ ID NO: 45 - DNA, 24 bp, Artificial Sequence
  Synthetic oligonucleotide
gccctcctgcacaagtttgacttt

SEQ ID NO: 46 - DNA, 24 bp, Artificial Sequence
  Synthetic oligonucleotide
agttggtctctgtgcaagcgtagt

SEQ ID NO: 47 - DNA, 20 bp, Artificial Sequence
  Synthetic oligonucleotide
gaatctcgaaatctcagccc

SEQ ID NO: 48 - DNA, 21 bp, Artificial Sequence
  Synthetic oligonucleotide
cttcactaatttgctcaggac

SEQ ID NO: 49 - DNA, 24 bp, Artificial Sequence
  Synthetic oligonucleotide
agcgaaactgtcagaggaggaaca

SEQ ID NO: 50 - DNA, 24 bp, Artificial Sequence
  Synthetic oligonucleotide
tcatgcagctggtacgtggtgaaa

SEQ ID NO: 51 - DNA, 24 bp, Artificial Sequence
  Synthetic oligonucleotide
cgagcagaagacgcattgcttcaa

SEQ ID NO: 52 - DNA, 24 bp, Artificial Sequence
  Synthetic oligonucleotide
cggccttggctatcatacatcaca

SEQ ID NO: 53 - DNA, 24 bp, Artificial Sequence
  Synthetic oligonucleotide
atttgggacggcgaacagaagaca

SEQ ID NO: 54 - DNA, 24 bp, Artificial Sequence
  Synthetic oligonucleotide
atcctggatgggcaactcagatgt

SEQ ID NO: 55 - DNA, 20 bp, Artificial Sequence
  Synthetic oligonucleotide
caatgcggggaggagaagtc

SEQ ID NO: 56 - DNA, 20 bp, Artificial Sequence
  Synthetic oligonucleotide
ctctggaccaaactgtggcg

SEQ ID NO: 57 - DNA, 18 bp, Artificial Sequence
  Synthetic oligonucleotide
cccccggcggcaatagca

SEQ ID NO: 58 - DNA, 20 bp, Artificial Sequence
  Synthetic oligonucleotide
tcggcgccggggagatacat

SEQ ID NO: 59 - DNA, 24 bp, Artificial Sequence
  Synthetic oligonucleotide
atggcaaattctgtggcgctgaag

SEQ ID NO: 60 - DNA, 24 bp, Artificial Sequence
  Synthetic oligonucleotide
gcgctgatttcccaagtgcattct